European Patent Application EP 4 722 369 A1, published April 8, 2026. Title: Protocatechuic acid-producing Hydrogenophilus bacterium transformant. Applicant: 株式会社ＣＯ２資源化研究所. The sequence listing filed with the application follows.

SEQUENCE LISTING (30 sequences)

SEQ ID NO: 1 - DNA, 1857 bp, Corynebacterium glutamicum
  source 1..1857: mol_type = genomic DNA
atgcgtacatccattgccactgtttgtttgtccggaactcttgctgaaaagctgcgcgcagctgcagatgctggatttgatggtgtggaaatcttcgagcaggacttggtggtttccccgcattcggcagagcagattcgtcagcgggctcaggatttgggattaaccctggatctgttccagccgtttcgagatttcgaaggtgtggaagaagagcagtttctgaagaatctgcaccgcttggaagagaagttcaagctgatgaacaggcttggcattgagatgatcttgttgtgttccaatgtgggcaccgcgaccatcaatgatgatgaccttttcgtggagcagttgcatcgtgcagcagatttggctgagaagtacaacgtcaagattgcttatgaagcgttggcgtggggcaagtttgtcaatgattttgagcatgcgcatgcacttgtggagaaggtgaatcacaaggcgctgggaacctgcttggatacgttccatattctttcccgtggttgggaaaccgacgaggtggagaacatccctgcggagaagatcttctttgttcagttagcggatgcgccgaagctgagcatggacattttgtcctggtcgcgtcaccaccgtgttttccctggtgaaggcgatttcgatctggtgaaattcatggttcatctggccaagacgggttatgatggcccgatttctttggagatcttcaacgattccttccgcaaggccgaggttggtcgcaccgcgattgatgggttgcgttctttgcgttggttggaagatcagacctggcatgcgctaaatgctgaggatcgtccaagcgctcttgaactgcgtgcacttcctgaggtcgcggaacctgagggtgttgatttcattgagatcgccactggacgtttgggtgagaccattcgggttcttcatcaattgggtttccgcttgggtggtcatcactgcagtaagcaggattaccaggtatggacccagggcgatgtgcgcattgtggtgtgtgatcgtggggtcaccggggctccaaccacgatctctgcgatgggctttgacacccccgatccagaagctgctcatgcccgtgcggaattgctgcgggctcagacaattgatcgtccccacatcgagggcgaagttgacctaaaaggtgtgtacgcaccggatggggtggagctgtttttcgcggggccgagccccgatggaatgcccgagtggctgccggaattcggcgtcgaaaagcaagaagctggtctcattgaagccatcgaccacgtcaatttcgcccagccgtggcaacattttgatgaggcagtgctgttttacaccgcgctgatggcgttggagactgtgcgtgaggatgagttcccgagcccaattggtttggtgcgcaatcaggtgatgcgttcgccgaatgatgcggtgcggttgctgctcagcgtggcgccggaggacggtgagcagggagatttcctcaacgcggcctacccggagcacattgcgttggccacggcggacatcgtggcggtggctgaacgtgcgcgcaaacgaggcctggatttcttgcccgtcccagagaattactacgacgatgtgcaggcgcgttttgatttgccgcaggaattcttggacacactcaaggaaaaccacctgctttacgaccgcgacgagaacggcgaattcctccacttttacacccgcacgttgggcacgctgttcttcgaagtggtggaacgccgcggcggttttgcaggttggggcgaaacaaacgctccggtgcggttggcggcgcagtatcgtgaggtgcgggacctcgagcggggaatcccaaactag

SEQ ID NO: 2 - protein, 618 aa, Corynebacterium glutamicum
MRTSIATVCLSGTLAEKLRAAADAGFDGVEIFEQDLVVSPHSAEQIRQRAQDLGLTLDLFQPFRDFEGVEEEQFLKNLHRLEEKFKLMNRLGIEMILLCSNVGTATINDDDLFVEQLHRAADLAEKYNVKIAYEALAWGKFVNDFEHAHALVEKVNHKALGTCLDTFHILSRGWETDEVENIPAEKIFFVQLADAPKLSMDILSWSRHHRVFPGEGDFDLVKFMVHLAKTGYDGPISLEIFNDSFRKAEVGRTAIDGLRSLRWLEDQTWHALNAEDRPSALELRALPEVAEPEGVDFIEIATGRLGETIRVLHQLGFRLGGHHCSKQDYQVWTQGDVRIVVCDRGVTGAPTTISAMGFDTPDPEAAHARAELLRAQTIDRPHIEGEVDLKGVYAPDGVELFFAGPSPDGMPEWLPEFGVEKQEAGLIEAIDHVNFAQPWQHFDEAVLFYTALMALETVREDEFPSPIGLVRNQVMRSPNDAVRLLLSVAPEDGEQGDFLNAAYPEHIALATADIVAVAERARKRGLDFLPVPENYYDDVQARFDLPQEFLDTLKENHLLYDRDENGEFLHFYTRTLGTLFFEVVERRGGFAGWGETNAPVRLAAQYREVRDLERGIPN

SEQ ID NO: 3 - DNA, 1911 bp, Pseudomonas thermotolerans
  source 1..1911: mol_type = genomic DNA
atgcagcgttcgatcgccaccgtctccctgagcggtacacttccggaaaaactcgaagccatagccgccgccggattcgacggcgtggagatattcgagaacgatctgctctactacgccggcagtccccgcgaagtgcgtcagctatgcgccgacctcggcctggccatcacgctgttccagccgtttcgcgacttcgagggctgccgtcgcgaccgcctggagaagaatctcgaccgcgccgagcgcaagttcgacctgatgcaggagctgggcaccgacctgattctggtgtgcagcaacgtggcaccggattccctgggcgatccgcgtatcatcgccgacgacctgcagcgcctcgcagagcgggccggcgctcgcggcctgcgcatcggctacgaggccctggcctggggccgccacgtgaacagctggcagcaggtttggaacatcgttcgcgaggtggaccaccccgccctcggcgtgttgctggacagcttccacaccctgtcgatccagggcgacccgagcggcatcgccgagattcccggcgacaggatcttcttcgtacagatggccgacgcgcccatcctggccatggatgtgctggagtggagccgccacttccgctgcttccccggacagggcgagttcgatctggccggcttcctggcgccgatcctgaagagcggctaccgcggcccgctgtccctggagatcttcaatgacggcttccgcgccgcgccgccgcgttccaatgccgccgacggcctgcgctcgctgctctacctggaggagaaaactcggcagcgcctggccgcggagggtagtccgctggccgagtcggagcaactgttcgcaccgccgcctgccagcccctacgagggcgtggagttcctcgagttcgccgtggacgaggagcagggtgcgcgcctggctagctggctggagaaactcggtttcgcccgcgtcggccgacaccgttccaaggaggtcagcctgctgcgccagggggatatcaacctggtgctcaacgccgagccctattccttcgcccgcaacttcttcgaggcccatggtccctcgttgtgcgccaccgcgctgcgggttcgcgaccaggctggcgccctggcccgcgcccagtccttcaggggccagccgttccgcggcctggtcggtcccaacgagaccgagatccccgcggtgcgtgccccggacggcagcctgatctatctggtggagcgcagtgcaccggggcagaccatctacgacaaggacttcctgctcgacgggcaggcccggcccagcggcagcctcaagcgcatcgaccacatggccgtggcgctgccggccgacagcctggatagctgggtgttgttctacaagagcctgttcgacttcgaggccgacgacgaggtggtgttacctgacccctacggcctggtgaagagccgggccatccgcagccgctgcagcaccgtgcgcctgccgctgaacatctcggagaaccgcaacacggcgatctcccacgcgctgtccagctaccgcggctccggcgtgcaccacatcgccttctcctgcgaggacctgttcgccgaggtgagccgcgccaaggacgccggagtgccgctgctggagatcccgctcaactactacgacgacctggccgcgcgtttcgacttcgacgacgaattcctcagcgagctggcctactacaacgtgctctacgatcgcgatgcccagggtggcgagctgttccacgtctacaccgagcctttcgaaggacgcttcttcttcgagctgctgcagcggcgcaacggctataccggctacggtgcggccaacgtcgccgtacgtctggccgcgctggccaagacgcgcagcggcgccgctcgtcagcccaggctctga

SEQ ID NO: 4 - protein, 636 aa, Pseudomonas thermotolerans
MQRSIATVSLSGTLPEKLEAIAAAGFDGVEIFENDLLYYAGSPREVRQLCADLGLAITLFQPFRDFEGCRRDRLEKNLDRAERKFDLMQELGTDLILVCSNVAPDSLGDPRIIADDLQRLAERAGARGLRIGYEALAWGRHVNSWQQVWNIVREVDHPALGVLLDSFHTLSIQGDPSGIAEIPGDRIFFVQMADAPILAMDVLEWSRHFRCFPGQGEFDLAGFLAPILKSGYRGPLSLEIFNDGFRAAPPRSNAADGLRSLLYLEEKTRQRLAAEGSPLAESEQLFAPPPASPYEGVEFLEFAVDEEQGARLASWLEKLGFARVGRHRSKEVSLLRQGDINLVLNAEPYSFARNFFEAHGPSLCATALRVRDQAGALARAQSFRGQPFRGLVGPNETEIPAVRAPDGSLIYLVERSAPGQTIYDKDFLLDGQARPSGSLKRIDHMAVALPADSLDSWVLFYKSLFDFEADDEVVLPDPYGLVKSRAIRSRCSTVRLPLNISENRNTAISHALSSYRGSGVHHIAFSCEDLFAEVSRAKDAGVPLLEIPLNYYDDLAARFDFDDEFLSELAYYNVLYDRDAQGGELFHVYTEPFEGRFFFELLQRRNGYTGYGAANVAVRLAALAKTRSGAARQPRL

SEQ ID NO: 5 - DNA, 35 bp, synthetic construct
  source 1..35: mol_type = other DNA
ttttataacccgggccatcgactgcacggtgcacc

SEQ ID NO: 6 - DNA, 35 bp, synthetic construct
  source 1..35: mol_type = other DNA
tgctagcactgtttcctgtgtgaaattgttatccg

SEQ ID NO: 7 - DNA, 38 bp, synthetic construct
  source 1..38: mol_type = other DNA
ggaaacagtgctagcagatctggaggagaaaggcatat

SEQ ID NO: 8 - DNA, 72 bp, synthetic construct
  source 1..72: mol_type = other DNA
cagtgcggccgcaagcttgtcgacggagctcgaattcggatccgatatcagcatatgcgtttctcctccaga

SEQ ID NO: 9 - DNA, 80 bp, synthetic construct
  source 1..80: mol_type = other DNA
acaagcttgcggccgcactgcagcaccatcaccaccatcattgataagatccggctgctaacaaagcccgaaaggaagct

SEQ ID NO: 10 - DNA, 63 bp, synthetic construct
  source 1..63: mol_type = other DNA
tatttgaatcgagttattgctcagcggtggcagcagccaactcagcttcctttcgggctttgt

SEQ ID NO: 11 - DNA, 35 bp, synthetic construct
  source 1..35: mol_type = other DNA
taactcgattcaaataaaacgaaaggctcagtcga

SEQ ID NO: 12 - DNA, 35 bp, synthetic construct
  source 1..35: mol_type = other DNA
cctagatccgcggagtttgtagaaacgcaaaaagg

SEQ ID NO: 13 - DNA, 35 bp, synthetic construct
  source 1..35: mol_type = other DNA
acaaactccgcggatctaggtgaagatcctttttg

SEQ ID NO: 14 - DNA, 35 bp, synthetic construct
  source 1..35: mol_type = other DNA
cgtccgcggccagcaaaaggccaggaaccgtaaaa

SEQ ID NO: 15 - DNA, 35 bp, synthetic construct
  source 1..35: mol_type = other DNA
ttgctggccgcggacgtagaaagcctgtccgcaga

SEQ ID NO: 16 - DNA, 35 bp, synthetic construct
  source 1..35: mol_type = other DNA
ggcccgggttataaaagccagtcattaggcctatc

SEQ ID NO: 17 - DNA, 35 bp, synthetic construct
  source 1..35: mol_type = other DNA
aattgtcagataggcctaatgactggcttttataa

SEQ ID NO: 18 - DNA, 35 bp, synthetic construct
  source 1..35: mol_type = other DNA
tgacgccagaagcattggtgcaccgtgcagtcgat

SEQ ID NO: 19 - DNA, 19 bp, synthetic construct
  source 1..19: mol_type = other DNA
gatctggaggagaaacgca

SEQ ID NO: 20 - DNA, 17 bp, synthetic construct
  source 1..17: mol_type = other DNA
tatgcgtttctcctcca

SEQ ID NO: 21 - DNA, 35 bp, synthetic construct
  source 1..35: mol_type = other DNA
gaggccatctaggccatgagtaagtctgacggaac

SEQ ID NO: 22 - DNA, 35 bp, synthetic construct
  source 1..35: mol_type = other DNA
atccggcacccatatctgaaccggacgcaaacccg

SEQ ID NO: 23 - DNA, 35 bp, synthetic construct
  source 1..35: mol_type = other DNA
ttcagatatgggtgccggatacccgccgcccgggc

SEQ ID NO: 24 - DNA, 35 bp, synthetic construct
  source 1..35: mol_type = other DNA
aaggccttcatggccttatttcgcgattcccaaga

SEQ ID NO: 25 - DNA, 43 bp, synthetic construct
  source 1..43: mol_type = other DNA
ctggaggagaaacgcatatgcgtacatccattgccactgtttg

SEQ ID NO: 26 - DNA, 44 bp, synthetic construct
  source 1..44: mol_type = other DNA
cgacggagctcgaattcctagtttgggattccccgctcgaggtc

SEQ ID NO: 27 - DNA, 43 bp, synthetic construct
  source 1..43: mol_type = other DNA
ctggaggagaaacgcatatgcagcgttcgatcgccaccgtctc

SEQ ID NO: 28 - DNA, 43 bp, synthetic construct
  source 1..43: mol_type = other DNA
cgacggagctcgaattctcagagcctgggctgacgagcggcgc

SEQ ID NO: 29 - DNA, 20 bp, synthetic construct
  source 1..20: mol_type = other DNA
gaattcgagctccgtcgaca

SEQ ID NO: 30 - DNA, 20 bp, synthetic construct
  source 1..20: mol_type = other DNA
atgcgtttctcctccagatc